European Patent Specification EP 3 526 332 B1, published June 26, 2024. Title: RECOMBINANT VIRUS REPLICON SYSTEMS AND USES THEREOF. Applicant: SYNTHETIC GENOMICS INC. The sequence listing filed with the application follows.

SEQUENCE LISTING (24 sequences)

SEQ ID NO: 1 - DNA, 8364 bp, Artificial Sequence
  Synthetic polynucleotide
  misc_feature: Rep-Alpha replicon
  misc_feature: T7 promoter, modified VEEV 5'UTR and nonstructural genes
taatacgactcactatagagaggcggcgcatgagagaagcccagaccaattacctacccaaaatggagaaagttcacgttgacatcgaggaagacagcccattcctcagagctttgcagcggagcttcccgcagtttgaggtagaagccaagcaggtcactgataatgaccatgctaatgccagagcgttttcgcatctggcttcaaaactgatcgaaacggaggtggacccatccgacacgatccttgacattggaagtgcgcccgcccgcagaatgtattctaagcacaagtatcattgtatctgtccgatgagatgtgcggaagatccggacagattgtataagtatgcaactaagctgaagaaaaactgtaaggaaataactgataaggaattggacaagaaaatgaaggagctcgccgccgtcatgagcgaccctgacctggaaactgagactatgtgcctccacgacgacgagtcgtgtcgctacgaagggcaagtcgctgtttaccaggatgtatacgcggttgacggaccgacaagtctctatcaccaagccaataagggagttagagtcgcctactggataggctttgacaccaccccttttatgtttaagaacttggctggagcatatccatcatactctaccaactgggccgacgaaaccgtgttaacggctcgtaacataggcctatgcagctctgacgttatggagcggtcacgtagagggatgtccattcttagaaagaagtatttgaaaccatccaacaatgttctattctctgttggctcgaccatctaccacgagaagagggacttactgaggagctggcacctgccgtctgtatttcacttacgtggcaagcaaaattacacatgtcggtgtgagactatagttagttgcgacgggtacgtcgttaaaagaatagctatcagtccaggcctgtatgggaagccttcaggctatgctgctacgatgcaccgcgagggattcttgtgctgcaaagtgacagacacattgaacggggagagggtctcttttcccgtgtgcacgtatgtgccagctacattgtgtgaccaaatgactggcatactggcaacagatgtcagtgcggacgacgcgcaaaaactgctggttgggctcaaccagcgtatagtcgtcaacggtcgcacccagagaaacaccaataccatgaaaaattaccttttgcccgtagtggcccaggcatttgctaggtgggcaaaggaatataaggaagatcaagaagatgaaaggccactaggactacgagatagacagttagtcatggggtgttgttgggcttttagaaggcacaagataacatctatttataagcgcccggatacccaaaccatcatcaaagtgaacagcgatttccactcattcgtgctgcccaggataggcagtaacacattggagatcgggctgagaacaagaatcaggaaaatgttagaggagcacaaggagccgtcacctctcattaccgccgaggacgtacaagaagctaagtgcgcagccgatgaggctaaggaggtgcgtgaagccgaggagttgcgcgcagctctaccacctttggcagctgatgttgaggagcccactctggaagccgatgtcgacttgatgttacaagaggctggggccggctcagtggagacacctcgtggcttgataaaggttaccagctacgatggcgaggacaagatcggctcttacgctgtgctttctccgcaggctgtactcaagagtgaaaaattatcttgcatccaccctctcgctgaacaagtcatagtgataacacactctggccgaaaagggcgttatgccgtggaaccataccatggtaaagtagtggtgccagagggacatgcaatacccgtccaggactttcaagctctgagtgaaagtgccaccattgtgtacaacgaacgtgagttcgtaaacaggtacctgcaccatattgccacacatggaggagcgctgaacactgatgaagaatattacaaaactgtcaagcccagcgagcacgacggcgaatacctgtacgacatcgacaggaaacagtgcgtcaagaaagaactagtcactgggctagggctcacaggcgagctggtggatcctcccttccatgaattcgcctacgagagtctgagaacacgaccagccgctccttaccaagtaccaaccataggggtgtatggcgtgccaggatcaggcaagtctggcatcattaaaagcgcagtcaccaaaaaagatctagtggtgagcgccaagaaagaaaactgtgcagaaattataagggacgtcaagaaaatgaaagggctggacgtcaatgccagaactgtggactcagtgctcttgaatggatgcaaacaccccgtagagaccctgtatattgacgaagcttttgcttgtcatgcaggtactctcagagcgctcatagccattataagacctaaaaaggcagtgctctgcggggatcccaaacagtgcggtttttttaacatgatgtgcctgaaagtgcattttaaccacgagatttgcacacaagtcttccacaaaagcatctctcgccgttgcactaaatctgtgacttcggtcgtctcaaccttgttttacgacaaaaaaatgagaacgacgaatccgaaagagactaagattgtgattgacactaccggcagtaccaaacctaagcaggacgatctcattctcacttgtttcagagggtgggtgaagcagttgcaaatagattacaaaggcaacgaaataatgacggcagctgcctctcaagggctgacccgtaaaggtgtgtatgccgttcggtacaaggtgaatgaaaatcctctgtacgcacccacctctgaacatgtgaacgtcctactgacccgcacggaggaccgcatcgtgtggaaaacactagccggcgacccatggataaaaacactgactgccaagtaccctgggaatttcactgccacgatagaggagtggcaagcagagcatgatgccatcatgaggcacatcttggagagaccggaccctaccgacgtcttccagaataaggcaaacgtgtgttgggccaaggctttagtgccggtgctgaagaccgctggcatagacatgaccactgaacaatggaacactgtggattattttgaaacggacaaagctcactcagcagagatagtattgaaccaactatgcgtgaggttctttggactcgatctggactccggtctattttctgcacccactgttccgttatccattaggaataatcactgggataactccccgtcgcctaacatgtacgggctgaataaagaagtggtccgtcagctctctcgcaggtacccacaactgcctcgggcagttgccactggaagagtctatgacatgaacactggtacactgcgcaattatgatccgcgcataaacctagtacctgtaaacagaagactgcctcatgctttagtcctccaccataatgaacacccacagagtgacttttcttcattcgtcagcaaattgaagggcagaactgtcctggtggtcggggaaaagttgtccgtcccaggcaaaatggttgactggttgtcagaccggcctgaggctaccttcagagctcggctggatttaggcatcccaggtgatgtgcccaaatatgacataatatttgttaatgtgaggaccccatataaataccatcactatcagcagtgtgaagaccatgccattaagcttagcatgttgaccaagaaagcttgtctgcatctgaatcccggcggaacctgtgtcagcataggttatggttacgctgacagggccagcgaaagcatcattggtgctatagcgcggcagttcaagttttcccgggtatgcaaaccgaaatcctcacttgaagagacggaagttctgtttgtattcattgggtacgatcgcaaggcccgtacgcacaatccttacaagctttcatcaaccttgaccaacatttatacaggttccagactccacgaagccggatgtgcaccctcatatcatgtggtgcgaggggatattgccacggccaccgaaggagtgattataaatgctgctaacagcaaaggacaacctggcggaggggtgtgcggagcgctgtataagaaattcccggaaagcttcgatttacagccgatcgaagtaggaaaagcgcgactggtcaaaggtgcagctaaacatatcattcatgccgtaggaccaaacttcaacaaagtttcggaggttgaaggtgacaaacagttggcagaggcttatgagtccatcgctaagattgtcaacgataacaattacaagtcagtagcgattccactgttgtccaccggcatcttttccgggaacaaagatcgactaacccaatcattgaaccatttgctgacagctttagacaccactgatgcagatgtagccatatactgcagggacaagaaatgggaaatgactctcaaggaagcagtggctaggagagaagcagtggaggagatatgcatatccgacgactcttcagtgacagaacctgatgcagagctggtgagggtgcatccgaagagttctttggctggaaggaagggctacagcacaagcgatggcaaaactttctcatatttggaagggaccaagtttcaccaggcggccaaggatatagcagaaattaatgccatgtggcccgttgcaacggaggccaatgagcaggtatgcatgtatatcctcggagaaagcatgagcagtattaggtcgaaatgccccgtcgaagagtcggaagcctccacaccacctagcacgctgccttgcttgtgcatccatgccatgactccagaaagagtacagcgcctaaaagcctcacgtccagaacaaattactgtgtgctcatcctttccattgccgaagtatagaatcactggtgtgcagaagatccaatgctcccagcctatattgttctcaccgaaagtgcctgcgtatattcatccaaggaagtatctcgtggaaacaccaccggtagacgagactccggagccatcggcagagaaccaatccacagaggggacacctgaacaaccaccacttataaccgaggatgagaccaggactagaacgcctgagccgatcatcatcgaagaggaagaagaggatagcataagtttgctgtcagatggcccgacccaccaggtgctgcaagtcgaggcagacattcacgggccgccctctgtatctagctcatcctggtccattcctcatgcatccgactttgatgtggacagtttatccatacttgacaccctggagggagctagcgtgaccagcggggcaacgtcagccgagactaactcttacttcgcaaagagtatggagtttctggcgcgaccggtgcctgcgcctcgaacagtattcaggaaccctccacatcccgctccgcgcacaagaacaccgtcacttgcacccagcagggcctgctcgagaaccagcctagtttccaccccgccaggcgtgaatagggtgatcactagagaggagctcgaggcgcttaccccgtcacgcactcctagcaggtcggtctcgagaaccagcctggtctccaacccgccaggcgtaaatagggtgattacaagagaggagtttgaggcgttcgtagcacaacaacaatgacggtttgatgcgggtgcatacatcttttcctccgacaccggtcaagggcatttacaacaaaaatcagtaaggcaaacggtgctatccgaagtggtgttggagaggaccgaattggagatttcgtatgccccgcgcctcgaccaagaaaaagaagaattactacgcaagaaattacagttaaatcccacacctgctaacagaagcagataccagtccaggaaggtggagaacatgaaagccataacagctagacgtattctgcaaggcctagggcattatttgaaggcagaaggaaaagtggagtgctaccgaaccctgcatcctgttcctttgtattcatctagtgtgaaccgtgccttttcaagccccaaggtcgcagtggaagcctgtaacgccatgttgaaagagaactttccgactgtggcttcttactgtattattccagagtacgatgcctatttggacatggttgacggagcttcatgctgcttagacactgccagtttttgccctgcaaagctgcgcagctttccaaagaaacactcctatttggaacccacaatacgatcggcagtgccttcagcgatccagaacacgctccagaacgtcctggcagctgccacaaaaagaaattgcaatgtcacgcaaatgagagaattgcccgtattggattcggcggcctttaatgtggaatgcttcaagaaatatgcgtgtaataatgaatattgggaaacgtttaaagaaaaccccatcaggcttactgaagaaaacgtggtaaattacattaccaaattaaaaggaccaaaagctgctgctctttttgcgaagacacataatttgaatatgttgcaggacataccaatggacaggtttgtaatggacttaaagagagacgtgaaagtgactccaggaacaaaacatactgaagaacggcccaaggtacaggtgatccaggctgccgatccgctagcaacagcgtatctgtgcggaatccaccgagagctggttaggagattaaatgcggtcctgcttccgaacattcatacactgtttgatatgtcggctgaagactttgacgctattatagccgagcacttccagcctggggattgtgttctggaaactgacatcgcgtcgtttgataaaagtgaggacgacgccatggctctgaccgcgttaatgattctggaagacttaggtgtggacgcagagctgttgacgctgattgaggcggctttcggcgaaatttcatcaatacatttgcccactaaaactaaatttaaattcggagccatgatgaaatctggaatgttcctcacactgtttgtgaacacagtcattaacattgtaatcgcaagcagagtgttgagagaacggctaaccggatcaccatgtgcagcattcattggagatgacaatatcgtgaaaggagtcaaatcggacaaattaatggcagacaggtgcgccacctggttgaatatggaagtcaagattatagatgctgtggtgggcgagaaagcgccttatttctgtggagggtttattttgtgtgactccgtgaccggcacagcgtgccgtgtggcagaccccctaaaaaggctgtttaagcttggcaaacctctggcagcagacgatgaacatgatgatgacaggagaagggcattgcatgaagagtcaacacgctggaaccgagtgggtattctttcagagctgtgcaaggcagtagaatcaaggtatgaaaccgtaggaacttccatcatagttatggccatgactactctagctagcagtgttaaatcattcagctacctgagaggggcccctataactctctacggctaacctgaatggactacgacatagtctagtccgccaagatatcatcgatacagcagcaattggcaagctgcttacatagaaggcgcgccgtttaaacggccggccttaattaagtaacgatacagcagcaattggcaagctgcttacatagaactcgcggcgattggcatgccgctttaaaatttttattttatttttcttttcttttccgaatcggattttgtttttaatatttcaaaaaaaaaaaaaaaaaaaaaaaaaaaaaaaaaaaaaaaacccctctctaaacggaggggtttttttcagcgtaactggactggccacagttaggcggccgcgcatgttcatcatcagtaacccgtatcgtgagcatcctctctcgtttcatcggtatcattacctccatgaacagaaatcccccttacacggaggcatcagtgaccaaacaggaaaaaaccgcccttaacatggcccgctttatcagaagccagacattaacgcttctggagaaactcaacgagctggacgcggatgaacaggcagacatctgtgaatcgcttcacgaccacgctgatgagctttaccgcagctgcctcgcgcgtttcggtgatgacggtgaaaacctctgacacatgcagctcccggagacggtcacagcttgtctgtaagcggatgccgggagcagacaagcccgtcagggcgcgtcagcgggtgttggcgggtgtcggggcgcagccatgacccagtcacgtagcgatagcggagtgtatactggcttaactatgcggcatcagagcagattgtactgagagtgcaccatatg

SEQ ID NO: 2 - DNA, 50 bp, Aura virus
  misc_feature: 5'UTR
atagcggacggactagtacttgtactacagaattaactgccgtgtgccgc

SEQ ID NO: 3 - DNA, 50 bp, Chikungunya virus
  misc_feature: 5'UTR
atggctgcgtgagacacacgtagcctaccagtttcttactgctctactct

SEQ ID NO: 4 - DNA, 50 bp, O'Nyong-Nyong virus
  misc_feature: 5'UTR
atagctgcgtgatacacacacgcagcttacgggtttcatactgctctact

SEQ ID NO: 5 - DNA, 50 bp, Bebaru virus
  misc_feature: 5'UTR
atggcggctgtgtgacacacgagccgtcgatttcaaccttcttgctccct

SEQ ID NO: 6 - DNA, 50 bp, Semliki Forest virus
  misc_feature: 5'UTR
atggcggatgtgtgacatacacgacgccaaaagattttgttccagctcct

SEQ ID NO: 7 - DNA, 50 bp, Mayaro virus
  misc_feature: 5'UTR
atggcgggcaagtgacacttgttccgccggtcgtctctaagctcttcctc

SEQ ID NO: 8 - DNA, 50 bp, Getah virus
  misc_feature: 5'UTR
atggcggacgtgtgacatcaccgttcgctctttctaggatcctttgctac

SEQ ID NO: 9 - DNA, 50 bp, Sagiyama virus; identical to SEQ ID NO: 8
  misc_feature: 5'UTR

SEQ ID NO: 10 - DNA, 50 bp, Ndumu virus
  misc_feature: 5'UTR
atggtgcggagttgagagacgaagcaccaaacaactacgcggctcaccat

SEQ ID NO: 11 - DNA, 50 bp, Middleburg virus
  misc_feature: 5'UTR
attggtggttacgtacacgtgccaccaccccccaccctccaagcgatcca

SEQ ID NO: 12 - DNA, 50 bp, Eastern equine encephalitis virus
  misc_feature: 5'UTR
atagggtacggtgtagaggcaaccaccctatttccacctatccaaaatgg

SEQ ID NO: 13 - DNA, 50 bp, Fort Morgan virus
  misc_feature: 5'UTR
atagggtatggtttagaggcgcctaccctacttaaccgatccaaacatgg

SEQ ID NO: 14 - DNA, 50 bp, Buggy Creek virus; identical to SEQ ID NO: 13
  misc_feature: 5'UTR

SEQ ID NO: 15 - DNA, 50 bp, Venezuelan equine encephalitis virus
  misc_feature: 5'UTR
atgggcggcgcaagagagaagcccaaaccaattacctacccaaaatggag

SEQ ID NO: 16 - DNA, 50 bp, Whataroa virus
  misc_feature: 5'UTR
attggcggcatagtacatactatataaaagaaacagccgaccaattgcac

SEQ ID NO: 17 - DNA, 50 bp, Sindbis virus
  misc_feature: 5'UTR
attgacggcgtagtacacactattgaatcaaacagccgaccaattgcact

SEQ ID NO: 18 - DNA, 50 bp, Bebaru virus
  misc_feature: 5'UTR
attggcggcgtagtacacactattgaatcaaacagccgaccaattgcact

SEQ ID NO: 19 - DNA, 9476 bp, Artificial Sequence
  Alpha-R-rFF-T2G
  misc_feature (1)..(18): T7 promoter
  misc_feature (20)..(20): T to G substitution
  misc_feature (9437)..(9476): Poly A
taatacgactcactatagagaggcggcgcatgagagaagcccagaccaattacctacccaaaatggagaaagttcacgttgacatcgaggaagacagcccattcctcagagctttgcagcggagcttcccgcagtttgaggtagaagccaagcaggtcactgataatgaccatgctaatgccagagcgttttcgcatctggcttcaaaactgatcgaaacggaggtggacccatccgacacgatccttgacattggaagtgcgcccgcccgcagaatgtattctaagcacaagtatcattgtatctgtccgatgagatgtgcggaagatccggacagattgtataagtatgcaactaagctgaagaaaaactgtaaggaaataactgataaggaattggacaagaaaatgaaggagctcgccgccgtcatgagcgaccctgacctggaaactgagactatgtgcctccacgacgacgagtcgtgtcgctacgaagggcaagtcgctgtttaccaggatgtatacgcggttgacggaccgacaagtctctatcaccaagccaataagggagttagagtcgcctactggataggctttgacaccaccccttttatgtttaagaacttggctggagcatatccatcatactctaccaactgggccgacgaaaccgtgttaacggctcgtaacataggcctatgcagctctgacgttatggagcggtcacgtagagggatgtccattcttagaaagaagtatttgaaaccatccaacaatgttctattctctgttggctcgaccatctaccacgagaagagggacttactgaggagctggcacctgccgtctgtatttcacttacgtggcaagcaaaattacacatgtcggtgtgagactatagttagttgcgacgggtacgtcgttaaaagaatagctatcagtccaggcctgtatgggaagccttcaggctatgctgctacgatgcaccgcgagggattcttgtgctgcaaagtgacagacacattgaacggggagagggtctcttttcccgtgtgcacgtatgtgccagctacattgtgtgaccaaatgactggcatactggcaacagatgtcagtgcggacgacgcgcaaaaactgctggttgggctcaaccagcgtatagtcgtcaacggtcgcacccagagaaacaccaataccatgaaaaattaccttttgcccgtagtggcccaggcatttgctaggtgggcaaaggaatataaggaagatcaagaagatgaaaggccactaggactacgagatagacagttagtcatggggtgttgttgggcttttagaaggcacaagataacatctatttataagcgcccggatacccaaaccatcatcaaagtgaacagcgatttccactcattcgtgctgcccaggataggcagtaacacattggagatcgggctgagaacaagaatcaggaaaatgttagaggagcacaaggagccgtcacctctcattaccgccgaggacgtacaagaagctaagtgcgcagccgatgaggctaaggaggtgcgtgaagccgaggagttgcgcgcagctctaccacctttggcagctgatgttgaggagcccactctggaagccgatgtcgacttgatgttacaagaggctggggccggctcagtggagacacctcgtggcttgataaaggttaccagctacgatggcgaggacaagatcggctcttacgctgtgctttctccgcaggctgtactcaagagtgaaaaattatcttgcatccaccctctcgctgaacaagtcatagtgataacacactctggccgaaaagggcgttatgccgtggaaccataccatggtaaagtagtggtgccagagggacatgcaatacccgtccaggactttcaagctctgagtgaaagtgccaccattgtgtacaacgaacgtgagttcgtaaacaggtacctgcaccatattgccacacatggaggagcgctgaacactgatgaagaatattacaaaactgtcaagcccagcgagcacgacggcgaatacctgtacgacatcgacaggaaacagtgcgtcaagaaagaactagtcactgggctagggctcacaggcgagctggtggatcctcccttccatgaattcgcctacgagagtctgagaacacgaccagccgctccttaccaagtaccaaccataggggtgtatggcgtgccaggatcaggcaagtctggcatcattaaaagcgcagtcaccaaaaaagatctagtggtgagcgccaagaaagaaaactgtgcagaaattataagggacgtcaagaaaatgaaagggctggacgtcaatgccagaactgtggactcagtgctcttgaatggatgcaaacaccccgtagagaccctgtatattgacgaagcttttgcttgtcatgcaggtactctcagagcgctcatagccattataagacctaaaaaggcagtgctctgcggggatcccaaacagtgcggtttttttaacatgatgtgcctgaaagtgcattttaaccacgagatttgcacacaagtcttccacaaaagcatctctcgccgttgcactaaatctgtgacttcggtcgtctcaaccttgttttacgacaaaaaaatgagaacgacgaatccgaaagagactaagattgtgattgacactaccggcagtaccaaacctaagcaggacgatctcattctcacttgtttcagagggtgggtgaagcagttgcaaatagattacaaaggcaacgaaataatgacggcagctgcctctcaagggctgacccgtaaaggtgtgtatgccgttcggtacaaggtgaatgaaaatcctctgtacgcacccacctctgaacatgtgaacgtcctactgacccgcacggaggaccgcatcgtgtggaaaacactagccggcgacccatggataaaaacactgactgccaagtaccctgggaatttcactgccacgatagaggagtggcaagcagagcatgatgccatcatgaggcacatcttggagagaccggaccctaccgacgtcttccagaataaggcaaacgtgtgttgggccaaggctttagtgccggtgctgaagaccgctggcatagacatgaccactgaacaatggaacactgtggattattttgaaacggacaaagctcactcagcagagatagtattgaaccaactatgcgtgaggttctttggactcgatctggactccggtctattttctgcacccactgttccgttatccattaggaataatcactgggataactccccgtcgcctaacatgtacgggctgaataaagaagtggtccgtcagctctctcgcaggtacccacaactgcctcgggcagttgccactggaagagtctatgacatgaacactggtacactgcgcaattatgatccgcgcataaacctagtacctgtaaacagaagactgcctcatgctttagtcctccaccataatgaacacccacagagtgacttttcttcattcgtcagcaaattgaagggcagaactgtcctggtggtcggggaaaagttgtccgtcccaggcaaaatggttgactggttgtcagaccggcctgaggctaccttcagagctcggctggatttaggcatcccaggtgatgtgcccaaatatgacataatatttgttaatgtgaggaccccatataaataccatcactatcagcagtgtgaagaccatgccattaagcttagcatgttgaccaagaaagcttgtctgcatctgaatcccggcggaacctgtgtcagcataggttatggttacgctgacagggccagcgaaagcatcattggtgctatagcgcggcagttcaagttttcccgggtatgcaaaccgaaatcctcacttgaagagacggaagttctgtttgtattcattgggtacgatcgcaaggcccgtacgcacaatccttacaagctttcatcaaccttgaccaacatttatacaggttccagactccacgaagccggatgtgcaccctcatatcatgtggtgcgaggggatattgccacggccaccgaaggagtgattataaatgctgctaacagcaaaggacaacctggcggaggggtgtgcggagcgctgtataagaaattcccggaaagcttcgatttacagccgatcgaagtaggaaaagcgcgactggtcaaaggtgcagctaaacatatcattcatgccgtaggaccaaacttcaacaaagtttcggaggttgaaggtgacaaacagttggcagaggcttatgagtccatcgctaagattgtcaacgataacaattacaagtcagtagcgattccactgttgtccaccggcatcttttccgggaacaaagatcgactaacccaatcattgaaccatttgctgacagctttagacaccactgatgcagatgtagccatatactgcagggacaagaaatgggaaatgactctcaaggaagcagtggctaggagagaagcagtggaggagatatgcatatccgacgactcttcagtgacagaacctgatgcagagctggtgagggtgcatccgaagagttctttggctggaaggaagggctacagcacaagcgatggcaaaactttctcatatttggaagggaccaagtttcaccaggcggccaaggatatagcagaaattaatgccatgtggcccgttgcaacggaggccaatgagcaggtatgcatgtatatcctcggagaaagcatgagcagtattaggtcgaaatgccccgtcgaagagtcggaagcctccacaccacctagcacgctgccttgcttgtgcatccatgccatgactccagaaagagtacagcgcctaaaagcctcacgtccagaacaaattactgtgtgctcatcctttccattgccgaagtatagaatcactggtgtgcagaagatccaatgctcccagcctatattgttctcaccgaaagtgcctgcgtatattcatccaaggaagtatctcgtggaaacaccaccggtagacgagactccggagccatcggcagagaaccaatccacagaggggacacctgaacaaccaccacttataaccgaggatgagaccaggactagaacgcctgagccgatcatcatcgaagaggaagaagaggatagcataagtttgctgtcagatggcccgacccaccaggtgctgcaagtcgaggcagacattcacgggccgccctctgtatctagctcatcctggtccattcctcatgcatccgactttgatgtggacagtttatccatacttgacaccctggagggagctagcgtgaccagcggggcaacgtcagccgagactaactcttacttcgcaaagagtatggagtttctggcgcgaccggtgcctgcgcctcgaacagtattcaggaaccctccacatcccgctccgcgcacaagaacaccgtcacttgcacccagcagggcctgctcgagaaccagcctagtttccaccccgccaggcgtgaatagggtgatcactagagaggagctcgaggcgcttaccccgtcacgcactcctagcaggtcggtctcgagaaccagcctggtctccaacccgccaggcgtaaatagggtgattacaagagaggagtttgaggcgttcgtagcacaacaacaatgacggtttgatgcgggtgcatacatcttttcctccgacaccggtcaagggcatttacaacaaaaatcagtaaggcaaacggtgctatccgaagtggtgttggagaggaccgaattggagatttcgtatgccccgcgcctcgaccaagaaaaagaagaattactacgcaagaaattacagttaaatcccacacctgctaacagaagcagataccagtccaggaaggtggagaacatgaaagccataacagctagacgtattctgcaaggcctagggcattatttgaaggcagaaggaaaagtggagtgctaccgaaccctgcatcctgttcctttgtattcatctagtgtgaaccgtgccttttcaagccccaaggtcgcagtggaagcctgtaacgccatgttgaaagagaactttccgactgtggcttcttactgtattattccagagtacgatgcctatttggacatggttgacggagcttcatgctgcttagacactgccagtttttgccctgcaaagctgcgcagctttccaaagaaacactcctatttggaacccacaatacgatcggcagtgccttcagcgatccagaacacgctccagaacgtcctggcagctgccacaaaaagaaattgcaatgtcacgcaaatgagagaattgcccgtattggattcggcggcctttaatgtggaatgcttcaagaaatatgcgtgtaataatgaatattgggaaacgtttaaagaaaaccccatcaggcttactgaagaaaacgtggtaaattacattaccaaattaaaaggaccaaaagctgctgctctttttgcgaagacacataatttgaatatgttgcaggacataccaatggacaggtttgtaatggacttaaagagagacgtgaaagtgactccaggaacaaaacatactgaagaacggcccaaggtacaggtgatccaggctgccgatccgctagcaacagcgtatctgtgcggaatccaccgagagctggttaggagattaaatgcggtcctgcttccgaacattcatacactgtttgatatgtcggctgaagactttgacgctattatagccgagcacttccagcctggggattgtgttctggaaactgacatcgcgtcgtttgataaaagtgaggacgacgccatggctctgaccgcgttaatgattctggaagacttaggtgtggacgcagagctgttgacgctgattgaggcggctttcggcgaaatttcatcaatacatttgcccactaaaactaaatttaaattcggagccatgatgaaatctggaatgttcctcacactgtttgtgaacacagtcattaacattgtaatcgcaagcagagtgttgagagaacggctaaccggatcaccatgtgcagcattcattggagatgacaatatcgtgaaaggagtcaaatcggacaaattaatggcagacaggtgcgccacctggttgaatatggaagtcaagattatagatgctgtggtgggcgagaaagcgccttatttctgtggagggtttattttgtgtgactccgtgaccggcacagcgtgccgtgtggcagaccccctaaaaaggctgtttaagcttggcaaacctctggcagcagacgatgaacatgatgatgacaggagaagggcattgcatgaagagtcaacacgctggaaccgagtgggtattctttcagagctgtgcaaggcagtagaatcaaggtatgaaaccgtaggaacttccatcatagttatggccatgactactctagctagcagtgttaaatcattcagctacctgagaggggcccctataactctctacggctaacctgaatggactacgacatagtctagtccgccaagatatcgcaccatggaaaatatggaaaacgacgagaacatcgtggtgggccccaagcccttctaccccatcgaggaaggcagcgccggcacccagctgcggaagtacatggaaagatacgccaagctgggcgccattgccttcaccaacgccgtgaccggcgtggactacagctacgccgagtacctggaaaagagctgctgcctgggcaaggctctgcagaactacggcctggtggtggacggccggatcgccctgtgcagcgagaactgcgaggaattcttcatccccgtgatcgccggcctgttcatcggcgtgggcgtggctcccaccaacgagatctacaccctgcgggagctggtgcacagcctgggcatcagcaagcccaccatcgtgttcagcagcaagaagggcctggacaaagtcatcaccgtgcagaaaaccgtgaccaccatcaagaccatcgtgatcctggacagcaaggtggactaccggggctaccagtgcctggacaccttcatcaagcggaacaccccccctggcttccaggccagcagcttcaagaccgtggaggtggaccggaaagaacaggtggccctgatcatgaacagcagcggcagcaccggcctgcccaagggcgtgcagctgacccacgagaacaccgtgacccggttcagccacgccagggaccccatctacggcaaccaggtgtcccccggcaccgccgtgctgaccgtggtgcccttccaccacggcttcggcatgttcaccaccctgggctacctgatctgcggcttccgggtggtgatgctgaccaagttcgacgaggaaaccttcctgaaaaccctgcaggactacaagtgcacctacgtgattctggtgcccaccctgttcgccatcctgaacaagagcgagctgctgaacaagtacgacctgagcaacctggtggagatcgccagcggcggagcccccctgagcaaagaagtgggagaggccgtcgccaggcggttcaatctgcccggcgtgcggcagggctacggcctgaccgagacaaccagcgccatcatcatcacccccgagggcgacgacaagcctggagccagcggcaaggtggtgcccctgttcaaggccaaagtgatcgacctggacaccaagaagagcctgggccccaacagacggggcgaagtgtgcgtgaagggccccatgctgatgaagggctacgtgaacaaccccgaggccaccaaagagctgatcgacgaagagggctggctgcacaccggcgacatcggctactacgacgaagagaagcacttcttcatcgtggaccggctgaagagcctgatcaagtacaagggctatcaggtgccccctgccgagctggaaagcgtcctgctgcagcaccccagcatcttcgacgccggcgtggccggggtgccagatcctgtggccggcgagctgcctggcgccgtggtggtgctggaatccggcaagaacatgaccgagaaagaagtgatggactacgtcgccagccaggtgtccaacgccaagcggctgagaggcggcgtgagattcgtggacgaagtgccaaagggcctgaccggcaagatcgacggcagggccatccgggagatcctgaagaaacccgtggccaagatgtgattaattgatcgatacagcagcaattggcaagctgcttacatagaaggcgcgccgtttaaacggccggccttaattaagtaacgatacagcagcaattggcaagctgcttacatagaactcgcggcgattggcatgccgctttaaaatttttattttatttttcttttcttttccgaatcggattttgtttttaatatttcaaaaaaaaaaaaaaaaaaaaaaaaaaaaaaaaaaaaaaaa

SEQ ID NO: 20 - DNA, 1647 bp, Artificial Sequence
  Synthetic polynucleotide
  misc_feature: Red Firefly reporter gene - rFF
atggaaaatatggaaaacgacgagaacatcgtggtgggccccaagcccttctaccccatcgaggaaggcagcgccggcacccagctgcggaagtacatggaaagatacgccaagctgggcgccattgccttcaccaacgccgtgaccggcgtggactacagctacgccgagtacctggaaaagagctgctgcctgggcaaggctctgcagaactacggcctggtggtggacggccggatcgccctgtgcagcgagaactgcgaggaattcttcatccccgtgatcgccggcctgttcatcggcgtgggcgtggctcccaccaacgagatctacaccctgcgggagctggtgcacagcctgggcatcagcaagcccaccatcgtgttcagcagcaagaagggcctggacaaagtcatcaccgtgcagaaaaccgtgaccaccatcaagaccatcgtgatcctggacagcaaggtggactaccggggctaccagtgcctggacaccttcatcaagcggaacaccccccctggcttccaggccagcagcttcaagaccgtggaggtggaccggaaagaacaggtggccctgatcatgaacagcagcggcagcaccggcctgcccaagggcgtgcagctgacccacgagaacaccgtgacccggttcagccacgccagggaccccatctacggcaaccaggtgtcccccggcaccgccgtgctgaccgtggtgcccttccaccacggcttcggcatgttcaccaccctgggctacctgatctgcggcttccgggtggtgatgctgaccaagttcgacgaggaaaccttcctgaaaaccctgcaggactacaagtgcacctacgtgattctggtgcccaccctgttcgccatcctgaacaagagcgagctgctgaacaagtacgacctgagcaacctggtggagatcgccagcggcggagcccccctgagcaaagaagtgggagaggccgtcgccaggcggttcaatctgcccggcgtgcggcagggctacggcctgaccgagacaaccagcgccatcatcatcacccccgagggcgacgacaagcctggagccagcggcaaggtggtgcccctgttcaaggccaaagtgatcgacctggacaccaagaagagcctgggccccaacagacggggcgaagtgtgcgtgaagggccccatgctgatgaagggctacgtgaacaaccccgaggccaccaaagagctgatcgacgaagagggctggctgcacaccggcgacatcggctactacgacgaagagaagcacttcttcatcgtggaccggctgaagagcctgatcaagtacaagggctatcaggtgccccctgccgagctggaaagcgtcctgctgcagcaccccagcatcttcgacgccggcgtggccggggtgccagatcctgtggccggcgagctgcctggcgccgtggtggtgctggaatccggcaagaacatgaccgagaaagaagtgatggactacgtcgccagccaggtgtccaacgccaagcggctgagaggcggcgtgagattcgtggacgaagtgccaaagggcctgaccggcaagatcgacggcagggccatccgggagatcctgaagaaacccgtggccaagatgtga

SEQ ID NO: 21 - DNA, 729 bp, Artificial Sequence
  Synthetic polynucleotide
  misc_feature: EGFP
atgggaagagccggcgtgagcaagggcgaggagctgttcaccggggtggtgcccatcctggtcgagctggacggcgacgtaaacggccacaagttcagcgtgtccggcgagggcgagggcgatgccacctacggcaagctgaccctgaagctgatctgcaccaccggcaagctgcccgtgccctggcccaccctcgtgaccaccctgggctacggcctgcagtgcttcgcccgctaccccgaccacatgaagcagcacgacttcttcaagtccgccatgcccgaaggctacgtccaggagcgcaccatcttcttcaaggacgacggcaactacaagacccgcgccgaggtgaagttcgagggcgacaccctggtgaaccgcatcgagctgaagggcatcgacttcaaggaggacggcaacatcctggggcacaagctggagtacaactacaacagccacaacgtctatatcaccgccgacaagcagaagaacggcatcaaggccaacttcaagatccgccacaacatcgaggacggcggcgtgcagctcgccgaccactaccagcagaacacccccatcggcgacggccccgtgctgctgcccgacaaccactacctgagctaccagtccgccctgagcaaagaccccaacgagaagcgcgatcacatggtcctgctggagttcgtgaccgccgccgggatcactctcggcatggacgagctgtacaag

SEQ ID NO: 22 - DNA, 1707 bp, Artificial Sequence
  Synthetic polynucleotide
  misc_feature: HA Influenza A virus A-VietNam-1203-2004 (H5N1) - GenBank
atggagaaaatagtgcttctttttgcaatagtcagtcttgttaaaagtgatcagatttgcattggttaccatgcaaacaactcgacagagcaggttgacacaataatggaaaagaacgttactgttacacatgcccaagacatactggaaaagaaacacaacgggaagctctgcgatctagatggagtgaagcctctaattttgagagattgtagcgtagctggatggctcctcggaaacccaatgtgtgacgaattcatcaatgtgccggaatggtcttacatagtggagaaggccaatccagtcaatgacctctgttacccaggggatttcaatgactatgaagaattgaaacacctattgagcagaataaaccattttgagaaaattcagatcatccccaaaagttcttggtccagtcatgaagcctcattaggggtgagctcagcatgtccataccagggaaagtcctcctttttcagaaatgtggtatggcttatcaaaaagaacagtacatacccaacaataaagaggagctacaataataccaaccaagaagatcttttggtactgtgggggattcaccatcctaatgatgcggcagagcagacaaagctctatcaaaacccaaccacctatatttccgttgggacatcaacactaaaccagagattggtaccaagaatagctactagatccaaagtaaacgggcaaagtggaaggatggagttcttctggacaattttaaagccgaatgatgcaatcaacttcgagagtaatggaaatttcattgctccagaatatgcatacaaaattgtcaagaaaggggactcaacaattatgaaaagtgaattggaatatggtaactgcaacaccaagtgtcaaactccaatgggggcgataaactctagcatgccattccacaatatacaccctctcaccattggggaatgccccaaatatgtgaaatcaaacagattagtccttgcgactgggctcagaaatagccctcaaagagagagaagaagaaaaaagagaggattatttggagctatagcaggttttatagagggaggatggcagggaatggtagatggttggtatgggtaccaccatagcaatgagcaggggagtgggtacgctgcagacaaagaatccactcaaaaggcaatagatggagtcaccaataaggtcaactcgatcattgacaaaatgaacactcagtttgaggccgttggaagggaatttaacaacttagaaaggagaatagagaatttaaacaagaagatggaagacgggttcctagatgtctggacttataatgctgaacttctggttctcatggaaaatgagagaactctagactttcatgactcaaatgtcaagaacctttacgacaaggtccgactacagcttagggataatgcaaaggagctgggtaacggttgtttcgagttctatcataaatgtgataatgaatgtatggaaagtgtaagaaatggaacgtatgactacccgcagtattcagaagaagcgagactaaaaagagaggaaataagtggagtaaaattggaatcaataggaatttaccaaatactgtcaatttattctacagtggcgagttccctagcactggcaatcatggtagctggtctatccttatggatgtgctccaatgggtcgttacaatgcagaatttgcatttaa

SEQ ID NO: 23 - DNA, 29 bp, Artificial Sequence
  Synthetic polynucleotide
  VEE 5' T-G nt 2 F - Forward Primer
cgactcactatagagaggcggcgcatgag

SEQ ID NO: 24 - DNA, 29 bp, Artificial Sequence
  Synthetic polynucleotide
  VEE 5' T-G nt 2 R - Reverse Primer
ctcatgcgccgcctctctatagtgagtcg